European Patent Application EP 4 491 633 A1, published January 15, 2025. Title: PD-L1-1-SPECIFIC CHIMERIC ANTIGEN RECEPTOR AND IMMUNE CELL COMPRISING SAME. Applicant: VAXCELL-BIO CO., LTD. Application EP 23767178.9, filed March 8, 2023. The sequence listing filed with the application follows.

SEQUENCE LISTING (16 sequences)

SEQ ID NO: 1 - DNA, 63 bp, synthetic construct
  misc_feature 1..63: note = CD8alpha signal sequence nucleotide
  source 1..63: mol_type = other DNA
atggccctgcctgtgacagctttgctgctgcctctggctctgctgctgcatgctgctagacct

SEQ ID NO: 2 - DNA, 765 bp, synthetic construct
  misc_feature 1..765: note = PD-L1 scFv nucleotide
  source 1..765: mol_type = other DNA
cagatgcagctggtgcagtctggggctgaggtgaagaagcctgggtcctcggtgaaggtctcctgcaaggcttctggaggcaccttcagcagctatgctatcagctgggtgcgacaggcccctggacaagggcttgagtggatgggaaggatcatccctatccttggtatagcaaactacgcacagaagttccagggcagagtcacgattaccgcggacaaatccacgagcacagcctacatggagctgagcagcctgagatctgaggacacggccgtgtattactgtgcgaaaccgagagatggctacaatttggttgcttttgatatctggggccaagggacgatggtcaccgtctcctcaggcctcgggggcctcggaggaggaggtagtggcggaggaggctccggtggatccagcggtgtgggttcccagctcgtgctgactcagccgccctcagtgtctggggccccagggcagagggtcaccatctcctgcactgggagcagctccaacatcggggcaggttatgatgtacactggtatcagcaacttccaggagcagcccccaaactcctcatctatggcgacatcaatcggccctcaggggtccctgaccgattctctggctccaagtctggcatctcagcctccctggctatcactgggctccaggctgaggacgaggctgattattactgccagtcctatgacagcagcctgagtgggggggtgttcggcggagggaccaagctgaccgtccta

SEQ ID NO: 3 - DNA, 207 bp, synthetic construct
  misc_feature 1..207: note = CD8alpha H and TM nucleotide
  source 1..207: mol_type = other DNA
accaccacaccagctccacggcctccaacaccagcacctacaattgcctctcagcccctgtctctgaggccagaagcttgtagacctgctgcaggcggagccgtgcataccagaggactggatttcgcctgcgacatctacatttgggcccctctggctggaacatgtggcgtcctgctgctgtctctcgtgatcaccctgtactgc

SEQ ID NO: 4 - DNA, 123 bp, synthetic construct
  misc_feature 1..123: note = CD28 nucleotide
  source 1..123: mol_type = other DNA
agaagcaagagaagccggctgctgcacagcgactacatgaacatgacccctagacggcccggacctaccagaaagcactaccagccttacgctcctcctcgggactttgccgcctatagatcc

SEQ ID NO: 5 - DNA, 126 bp, synthetic construct
  misc_feature 1..126: note = 4-1BB nucleotide
  source 1..126: mol_type = other DNA
aagcggggcagaaagaagctgctgtacatcttcaagcagcccttcatgcggcccgtgcagaccacacaagaggaagatggctgctcctgcagattccccgaggaagaagaaggcggctgcgagctg

SEQ ID NO: 6 - DNA, 339 bp, synthetic construct
  misc_feature 1..339: note = CD3zeta nucleotide
  source 1..339: mol_type = other DNA
agagtgaagttctctagatctgccgacgctcctgcctaccagcagggacagaatcagctgtacaacgagctgaatctggggcgcagagaagagtacgacgtgctggataagagaagaggcagagatcccgagatgggcggcaagccccagagaagaaagaatccccaagagggcctgtataatgagctgcagaaagacaagatggccgaggcctacagcgagatcggaatgaagggcgaacgcagaagaggaaagggccacgacggactgtatcagggcctgagcacagccaccaaggatacctatgatgccctgcacatgcaggccctgccacctagg

SEQ ID NO: 7 - protein, 21 aa, synthetic construct
  REGION 1..21: note = CD8alpha signal sequence amino acid
MALPVTALLLPLALLLHAARP

SEQ ID NO: 8 - protein, 255 aa, synthetic construct
  REGION 1..255: note = PD-L1 scFv amino acid
QMQLVQSGAEVKKPGSSVKVSCKASGGTFSSYAISWVRQAPGQGLEWMGRIIPILGIANYAQKFQGRVTITADKSTSTAYMELSSLRSEDTAVYYCAKPRDGYNLVAFDIWGQGTMVTVSSGLGGLGGGGSGGGGSGGSSGVGSQLVLTQPPSVSGAPGQRVTISCTGSSSNIGAGYDVHWYQQLPGAAPKLLIYGDINRPSGVPDRFSGSKSGISASLAITGLQAEDEADYYCQSYDSSLSGGVFGGGTKLTVL

SEQ ID NO: 9 - protein, 69 aa, synthetic construct
  REGION 1..69: note = CD8alpha H and TM amino acid
TTTPAPRPPTPAPTIASQPLSLRPEACRPAAGGAVHTRGLDFACDIYIWAPLAGTCGVLLLSLVITLYC

SEQ ID NO: 10 - protein, 41 aa, synthetic construct
  REGION 1..41: note = CD28 amino acid
RSKRSRLLHSDYMNMTPRRPGPTRKHYQPYAPPRDFAAYRS

SEQ ID NO: 11 - protein, 42 aa, synthetic construct
  REGION 1..42: note = 4-1BB amino acid
KRGRKKLLYIFKQPFMRPVQTTQEEDGCSCRFPEEEEGGCEL

SEQ ID NO: 12 - protein, 113 aa, synthetic construct
  REGION 1..113: note = CD3zeta amino acid
RVKFSRSADAPAYQQGQNQLYNELNLGRREEYDVLDKRRGRDPEMGGKPQRRKNPQEGLYNELQKDKMAEAYSEIGMKGERRRGKGHDGLYQGLSTATKDTYDALHMQALPPR

SEQ ID NO: 13 - DNA, 17 bp, synthetic construct
  misc_feature 1..17: note = CPL F
  source 1..17: mol_type = other DNA
accaccacaccagctcc

SEQ ID NO: 14 - DNA, 18 bp, synthetic construct
  misc_feature 1..18: note = CPL R
  source 1..18: mol_type = other DNA
aggtctagcagcatgcag

SEQ ID NO: 15 - DNA, 36 bp, synthetic construct
  misc_feature 1..36: note = VYPC F
  source 1..36: mol_type = other DNA
ctgcatgctgctagacctcagatgcagctggtgcag

SEQ ID NO: 16 - DNA, 38 bp, synthetic construct
  misc_feature 1..38: note = VYPC R
  source 1..38: mol_type = other DNA
tggagctggtgtggtggttaggacggtcagcttggtcc